European Patent Application EP 4 544 920 A1, published April 30, 2025. Title: METHOD FOR PREPARING, AND INCREASING FLAVOR MOLECULES IN, YEAST EXTRACT AND USE OF THE YEAST EXTRACT. Applicant: National Chung Hsing University. The sequence listing filed with the application follows.

SEQUENCE LISTING (35 sequences)

SEQ ID NO: 1 - protein, 9 aa, Kluyveromyces sp.
PPPPPPPPP

SEQ ID NO: 2 - protein, 10 aa, Kluyveromyces sp.
GPPPPPPPPP

SEQ ID NO: 3 - protein, 11 aa, Kluyveromyces sp.
GPPPPPPPPPA

SEQ ID NO: 4 - protein, 11 aa, Kluyveromyces sp.
DVPVVPGTPGP

SEQ ID NO: 5 - protein, 7 aa, Kluyveromyces sp.
DIPVPKP

SEQ ID NO: 6 - protein, 7 aa, Kluyveromyces sp.
DLPVPKP

SEQ ID NO: 7 - protein, 9 aa, Kluyveromyces sp.
VGDDVAVGR

SEQ ID NO: 8 - protein, 9 aa, Kluyveromyces sp.
DLQNPPPPP

SEQ ID NO: 9 - protein, 9 aa, Kluyveromyces sp.
KGDWPLDTK

SEQ ID NO: 10 - protein, 10 aa, Kluyveromyces sp.
DLQNPPPPPS

SEQ ID NO: 11 - protein, 12 aa, Kluyveromyces sp.
IIAEPWTIVGGK

SEQ ID NO: 12 - protein, 8 aa, Kluyveromyces sp.
DTKLPLVG

SEQ ID NO: 13 - protein, 8 aa, Kluyveromyces sp.
VDEPAVRE

SEQ ID NO: 14 - protein, 14 aa, Kluyveromyces sp.
GLDPPASPDDPTPE

SEQ ID NO: 15 - protein, 7 aa, Kluyveromyces sp.
EDDVVKL

SEQ ID NO: 16 - protein, 8 aa, Kluyveromyces sp.
LDDELKPT

SEQ ID NO: 17 - protein, 7 aa, Kluyveromyces sp.
FDDLIEE

SEQ ID NO: 18 - protein, 7 aa, Kluyveromyces sp.
MELITEE

SEQ ID NO: 19 - protein, 9 aa, Kluyveromyces sp.
IEEEGIALR

SEQ ID NO: 20 - protein, 9 aa, Kluyveromyces sp.
LGDDIEDRE

SEQ ID NO: 21 - protein, 8 aa, Kluyveromyces sp.
IDDDITRM

SEQ ID NO: 22 - protein, 8 aa, Kluyveromyces sp.
IDDEIVKT

SEQ ID NO: 23 - protein, 11 aa, Kluyveromyces sp.
LDDELKPTKPS

SEQ ID NO: 24 - protein, 13 aa, Kluyveromyces sp.
DEGKDIDIPNLVE

SEQ ID NO: 25 - protein, 8 aa, Kluyveromyces sp.
VDEPAVRE

SEQ ID NO: 26 - protein, 10 aa, Kluyveromyces sp.
VDDIIDRLLE

SEQ ID NO: 27 - protein, 12 aa, Kluyveromyces sp.
ENDAPIVEPVFE

SEQ ID NO: 28 - protein, 7 aa, Kluyveromyces sp.
DDGTLKL

SEQ ID NO: 29 - protein, 7 aa, Kluyveromyces sp.
DDGTIKI

SEQ ID NO: 30 - protein, 9 aa, Kluyveromyces sp.
VGDDVAVGR

SEQ ID NO: 31 - protein, 11 aa, Kluyveromyces sp.
NDAPIVEPVFE

SEQ ID NO: 32 - protein, 8 aa, Kluyveromyces sp.
DDGTLKLN

SEQ ID NO: 33 - protein, 8 aa, Kluyveromyces sp.
IGEPIDER

SEQ ID NO: 34 - protein, 8 aa, Kluyveromyces sp.
GGDEGRLF

SEQ ID NO: 35 - protein, 8 aa, Kluyveromyces sp.
LPDEPIDK